European Patent Application EP 4 715 049 A1, published March 25, 2026. Title: 보존된 잔기를 포함하는, PET 분해 활성을 갖는 폴리펩티드. Applicant: 주식회사 자이엔. Application KR. The sequence listing filed with the application follows.

SEQUENCE LISTING (2 sequences)

SEQ ID NO: 1 - protein, 365 aa, synthetic construct
  source 1..365: note = COG4188
AIFAAIGLREIAAAPVGVANLLADADLRQPGPEGVALFVTITLNDPQRDRERPVDLRLPQGGTGTVALYLLPLVVLSHGSGSYVTGFAWLAEHLASYGFVVAAPDHPGSNAGGAPAAYAGPGSYAPAEWWERPLDISALLDALLQLTASPALAGRLDPQRVGVLGHSFGGYTAMELAGAELDAEALLQHCESASRICLDPPGLNGRLLNQCAAVWLPRQAYDLRDPRIRAVVAINPALGMIFGTTGLVKVTDPVLLAAGSADGFAPPVTEQIRPFGYLPGALKYLRLVPGATHFSFLELCKEGQDIAAYTYRKSAALALAGLYVPICEEAGGFDRAAYAQLISTRVLPFFDVTLKTPAALFQQRQ

SEQ ID NO: 2 - protein, 447 aa, synthetic construct
  source 1..447: note = WP_039906502.1
MSPRFRGRLFKLAAAGIAAAVGMFTMTVATGSASAADNPYQRGPDPTRTSVTAVNGPFANTSVSVPTGYGFNGGRIYYPTDTSQGTFGAIAISPGYTALFSAELAWMGPWLASHGFVVIGIETNSRNDFDTARGTQLLAALDYLTQQSPVRDRVDPTRLAVAGHSMGGGGALSAATRRSSLKAAVGIAPYSPSSNLANDRVPTMVFAGQADTVVTPSYATGLYNSLPATTESAYLEVAGADHGFMVGRSNPVLVRTMLPFVKMFVDNDARYSQFLCPLLDSSGVVTYRSTCPLLPSTPTTPTATPTNTPTPTASPTVPPTSASQIVGTQSGRCVDVPNASRTNGTRVTLYDCNRQINQTWTYTANKQLQVYGTMCLDAAGTGNGAAVQIYNCHGQTNQQWNVNSNGTISSVQSGRCLDVWSTSNGAQIQLYDCHGQPNQQFRLVSLA